European Patent Specification EP 3 512 962 B1, published February 11, 2026. Title: DNA Degradation. Applicant: Qiagen GmbH. The sequence listing filed with the application follows.

SEQUENCE LISTING (47 sequences)

SEQ ID NO: 1 - DNA, 24 bp, Artificial Sequence
  primer
cctgaggatgccacagtgagacac

SEQ ID NO: 2 - DNA, 28 bp, Artificial Sequence
  primer
acttctgtctactgtcggactctacagg

SEQ ID NO: 3 - DNA, 24 bp, Artificial Sequence
  primer
ggcccagctttgacttgagaacag

SEQ ID NO: 4 - DNA, 24 bp, Artificial Sequence
  probe
tctggagggtccactgtgaggcag

SEQ ID NO: 5 - DNA, 24 bp, Artificial Sequence
  probe
tccaggcccagctcttgcctcatg

SEQ ID NO: 6 - DNA, 91 bp, Homo sapiens
cctgaggatgccacagtgagacaccatctgggtctggagggtccactgtgaggcagaggctggcctgtagagtccgacagtagacagaagt

SEQ ID NO: 7 - DNA, 91 bp, Homo sapiens
cctgaggatgccacagtgagacaccatctgggtctggagggtccactgtgaggcagaggctgacctgtagagtccgacagtagacagaagt

SEQ ID NO: 8 - DNA, 91 bp, Homo sapiens; identical to SEQ ID NO: 7

SEQ ID NO: 9 - DNA, 91 bp, Homo sapiens; identical to SEQ ID NO: 7

SEQ ID NO: 10 - DNA, 91 bp, Homo sapiens; identical to SEQ ID NO: 6

SEQ ID NO: 11 - DNA, 91 bp, Homo sapiens; identical to SEQ ID NO: 6

SEQ ID NO: 12 - DNA, 91 bp, Homo sapiens; identical to SEQ ID NO: 7

SEQ ID NO: 13 - DNA, 91 bp, Homo sapiens; identical to SEQ ID NO: 7

SEQ ID NO: 14 - DNA, 91 bp, Homo sapiens; identical to SEQ ID NO: 7

SEQ ID NO: 15 - DNA, 91 bp, Homo sapiens
cctgaggatgccacagtgagacaccatctgggtctgcagggtccactgtgaggcagaggctggcctgtagagtccgacagtagacacaagt

SEQ ID NO: 16 - DNA, 91 bp, Homo sapiens; identical to SEQ ID NO: 6

SEQ ID NO: 17 - DNA, 91 bp, Homo sapiens; identical to SEQ ID NO: 6

SEQ ID NO: 18 - DNA, 91 bp, Homo sapiens; identical to SEQ ID NO: 6

SEQ ID NO: 19 - DNA, 91 bp, Homo sapiens; identical to SEQ ID NO: 7

SEQ ID NO: 20 - DNA, 91 bp, Homo sapiens; identical to SEQ ID NO: 6

SEQ ID NO: 21 - DNA, 91 bp, Homo sapiens; identical to SEQ ID NO: 6

SEQ ID NO: 22 - DNA, 91 bp, Homo sapiens; identical to SEQ ID NO: 6

SEQ ID NO: 23 - DNA, 91 bp, Homo sapiens; identical to SEQ ID NO: 7

SEQ ID NO: 24 - DNA, 91 bp, Homo sapiens
actgaggatgccacagtgagacaccatctgggtctggagggtccactgtgaggcagaggctggcctgtagagtccgacagtagacagaagt

SEQ ID NO: 25 - DNA, 91 bp, Homo sapiens; identical to SEQ ID NO: 6

SEQ ID NO: 26 - DNA, 91 bp, Homo sapiens; identical to SEQ ID NO: 6

SEQ ID NO: 27 - DNA, 353 bp, Homo sapiens
cctgaggatgccacagtgagacaccatctgggtctggagggtccactgtgaggcagaggctggcctgtagagtccgacagtagacagaagttgggcaaaaggctgatttgaggaagttttgggcttcaagagtcagccacgaggcaggcactaggcctggaaatggcctgacagtcatgagttgggcctaaatgggccactgtgagggaggagctgtgcctgttgaggctgctggcaggcaggcagaaattcggcctggggcagctgccatgaggcaagagctgggcctggaaaaagcccctgggaggcaagagcagggcctgcagaggctgttctcaagtcaaagctgggcc

SEQ ID NO: 28 - DNA, 353 bp, Homo sapiens
cctgaggatgccacagtgagacaccatctgggtctggagggtccactgtgaggcagaggctgacctgtagagtccgacagtagacagaagttgggcaaaaggctgatttgaggaagttttgggcttcaagagtcagccacgaggcaggcactaggcctggaaatggcctcacagtcatgagttgggcctaaatgggccactgtgagggaggagctgtgcctgttgaggctgctggcaggcaggcagaaatttggcctggggcagccgccatgaggcaagagctgggcctggaaaaagcccctgggaggcaagagcagggcctgcagaggctgttctcaagtcaaagctgggcc

SEQ ID NO: 29 - DNA, 353 bp, Homo sapiens
cctgaggatgccacagtgagacaccatctgggtctggagggtccactgtgaggcagaggctgacctgtagagtccgacagtagacagaagttgggcaaaagcctgatttgaggaagttttgggcttcaagagtcagccacgaggcaggcactaggcctggaaatggcctcacagtcatgagttgggcctaaatgggccactgtgagggaggagctgtgcctgttgaggctgctggcaggcaggcagaaatttggcctggggcagctgccatgaggcaagagctgggcctggaaaaagcccctgggaggcaagagcagggcctgcagaggctgttctcaagtcaaagctgggcc

SEQ ID NO: 30 - DNA, 353 bp, Homo sapiens; identical to SEQ ID NO: 28

SEQ ID NO: 31 - DNA, 353 bp, Homo sapiens; identical to SEQ ID NO: 27

SEQ ID NO: 32 - DNA, 353 bp, Homo sapiens
cctgaggatgccacagtgagacaccatctgggtctggagggtccactgtgaggcagaggctggcctgtagagtccgacagtagacagaagttgggcaaaaggctgatttgaggaagttttgggcttcaagagtcagccacgaggcaggcactaggcctggaaatggcccgacagtcatgagttgggactaaatgggccactgtgagggaggagctgtgcctgttgaggctgctggcaggcaagcagaaatttggcctcgggcagctgccatgaggcaagagctgggcctggaaaaagcccctgggaggcaagagcagggcctgcagaggctgttctcaagtcaaagctgggcc

SEQ ID NO: 33 - DNA, 353 bp, Homo sapiens
cctgaggatgccacagtgagacaccatctgggtctggagggtccactgtgaggcagaggctgacctgtagagtccgacagtagacagaagttgggcaaaagcctgatttgaggaagttttgggcttcaagagtcagccacgaggcaggcactaggcctggaaatggactcacagtcatgagttgggcctaaatgggccactgtgagggaggagctgtgcctgttgaggctgctggcaggcaggcagaaatttggcctggggcagctgccatgaggcaagagctgggcctggaaaaagcccctgggaggcaagagcagggcctgcagaggctgttctcaagtcaaagctgggcc

SEQ ID NO: 34 - DNA, 353 bp, Homo sapiens; identical to SEQ ID NO: 29

SEQ ID NO: 35 - DNA, 353 bp, Homo sapiens
cctgaggatgccacagtgagacaccatctgggtctggagggtccactgtgaggcagaggctgacctgtagagtccgacagtagacagaagttgggcaaaagcctgatttgaggaagttttgggcttcaagagtcagccacgaggcaggcactaggcctggaaatggcctcacagtcataagttgggcctaaatgggccactgtgagggaggagctgtgcctgttgaggctgctggcaggcaggcagaaatttggcctggggcagctgccatgaggcaagagctgggcctggaaaaagcccctgggaggcaagagcagggcctgcagaggctgttctcaagtcaaagctgggcc

SEQ ID NO: 36 - DNA, 352 bp, Homo sapiens
cctgaggatgccacagtgagacaccatctgggtctgcagggtccactgtgaggcagaggctggcctgtagagtccgacagtagacacaagttgggcaaaaggctgatttgaggaagttttgggcttcaagagtcagccaggaggcaggcactaggcctggaaatggcccgacagtcatgagttgggcctaaatgggccaccgtgagggaggagctgtgcctgttgaggctgctggcaggcaggaagaaatttggcctgaggcagctgccatgaggcaagagctgggcttggaaaagcccctgggaggcaagagcaggccctgcagaggctgttctcaagtcaaagctgggcc

SEQ ID NO: 37 - DNA, 352 bp, Homo sapiens
cctgaggatgccacagtgagacaccatctgggtctggagggtccactgtgaggcagaggctggcctgtagagtccaacagtagacagaagttgagcaaaaggctaatttcaggaagttttgggcttcaagagtcagccaggaggcaggcactaggcctggaaatggcccgacagtcatgagttgggcctaaatgggccactgtgagggaggagctgtgcctgttgaggctgctggcaggcaggcagaaacttggcctggggcagctgccatgagacaagagctgggcctggagaagcccctgagaggtaagagcagggcctgcagaggctgttctcaagtcaaagctgggcc

SEQ ID NO: 38 - DNA, 352 bp, Homo sapiens
cctgaggatgccacagtgagacaccatctgggtctggagggtccactgtgaggcagaggctggcctgtagagtccgacagtagacagaagttgggcaaaaggctgatttgaggaagttttgggcttcaagagtcagccaggaggcaggcactaggcctggaaatggcccgacagtcatgagttgggcctaaatgggccactgtgagggaggagctgtgcctgttgaggctgctggcaggcaggcagaaacttggcctggggcagccgccatgaggcaagagctgggcctggagaagcccctgggaggcaagagcacggcctgcagaggctgttctcaagtcaaagctgggcc

SEQ ID NO: 39 - DNA, 352 bp, Homo sapiens; identical to SEQ ID NO: 38

SEQ ID NO: 40 - DNA, 353 bp, Homo sapiens
cctgaggatgccacagtgagacaccatctgggtctggagggtccactgtgaggcagaggctgacctgtagagtccgacagtagacagaagttgggcaaaaggctgatttgaggaagttttgggcttcaagagtcagccacgaggcaggcactaggcctggaaatggcctcacagtcatgagttgggcctaaatgggccactgtgagggaggagctgtgcctgttgaggctgctggcaggcaggcagaaatttggcctggggcagctgccatgaggcaagagctgggcctggaaaaagcccctgggaggcaagagcagggcctgcagaggctgttctcaagtcaaagctgggcc

SEQ ID NO: 41 - DNA, 352 bp, Homo sapiens
cctgaggatgccacagtgagacaccatctgagtctggagggtccactgtgaggcagaggctggcctgtagagtccaacagtagacagaagttgggcaaaaggctgatttgaggaagttttgggcttcaagagtcagccacgaggcaggcactaggcctggaaatggcctcacagtcatgagttgggcctaaatgggccactgtgagggaggagctgtgcctgttgaggctgctggcaggcaggcagaaatttggcctgggcagctgccacgaggcaagagctgggcctggaaaaagcccctgggaggcaagagcagggcctgcagaggctgttctcaagtcaaagctgggcc

SEQ ID NO: 42 - DNA, 353 bp, Homo sapiens
cctgaggatgccacagtgagacaccatctgggtctggagggtccactgtgaggcagaggctggcctgtagagtccgacagtagacagaagttgggcaaaaggctgatttgaggaagttttgggcttcaagagtcagccacgaggcaggcactaggcctggaaatggcccgacagtcatgagttgggcctaaatgggccactgtgagggaggagctgtgcctgttgaggctgctggcaggcaggcagaaatttggcctggggcagctgccatgaggcaggagctgggtctggaaaaagcccctgggaggcaagagcagggcctgcagaggctgttctcaagtcaaagctgggcc

SEQ ID NO: 43 - DNA, 356 bp, Homo sapiens
cctgaggatgccacagtgagacaccatctgggtctggagggtccactgtgaggcagaggctggcctgtagagtccgacagtagacagaagttaggcaaaaggctgatttgaggaagttttgggcttcaagaaagagtcagccaggaggcaggcactaggcctggaaatggcccgacagtcatgagtggggcctaaatgggccactgtgagggaggagctgtgcctgttgaggctgctggcaggcaggaagaaatttggcctggggcagctgccatgaggcaagagctgggcttggaaaagcccctgggaggcaagagcagggcctgcagaggctgttctcaagtcaaagctgggcc

SEQ ID NO: 44 - DNA, 353 bp, Homo sapiens; identical to SEQ ID NO: 29

SEQ ID NO: 45 - DNA, 353 bp, Homo sapiens
actgaggatgccacagtgagacaccatctgggtctggagggtccactgtgaggcagaggctggcctgtagagtccgacagtagacagaagttgggcaaaaggctgatttgaggaagttttgggcttcaagagtcagccacgaggcaggcactaggcctggaaatggcccgacagtcatgagttgggcctaaatgggccactgtgagggaggagctatgcctgttgaggctgctggcaggcaggcagaaatttggcctggggcagctgccatgaggcaagagctgggcctggaaaaagcccctgggaggcaagagcagggcctgcagaggctgttctcaagtcaaagctgggcc

SEQ ID NO: 46 - DNA, 352 bp, Homo sapiens
cctgaggatgccacagtgagacaccatctgggtctggagggtccactgtgaggcagaggctggcctgtagagtccgacagtagacagaagttgagcaaaaggctaatttcaggaagttttgggcttcaagagtcagccaggaggcaggcactaggcctggaaatggcccgacagtcatgagttgggcctaaatgggccactgtgagggaggagctgtgcctgttgaggctgctggcaggcaggcagaaacttggcctggagcagcttccatgagacaagagctgggcctggagaagcccctgagaggtaagaggagggcctgcagaggctgttctcaagtcaaagctgggcc

SEQ ID NO: 47 - DNA, 352 bp, Homo sapiens
cctgaggatgccacagtgagacaccatctgggtctggagggtccactgtgaggcagaggctggcctgtagagtccgacagtagacagaagttgggcaaaaggctgatttgaggaagttttgggcttcaagagtcagccaggaggcaggcactaggcctggaaatggcccgacagtcatgagttgggcctaaatgggccactgtgagggaagagctgtgcctgttgaggctgctggcaggcaggcagaaacttggcctggggcagccgccatgaggcaagagctgggcctggagaagcccctgggaggcaagagcagggcctgcagaggctgttctcaagtcaaagctgggcc